European Patent Specification EP 2 789 383 B1, published May 3, 2023. Title: Improvements in or relating to molecular assays. Applicant: Illumina Cambridge Limited. The sequence listing filed with the application follows.

SEQUENCE LISTING (9 sequences)

SEQ ID NO: 1 - DNA, 31 bp, Artificial Sequence
  Primer sequence
ttttttttttcaagcagaagacggcatacga

SEQ ID NO: 2 - DNA, 30 bp, Artificial Sequence
  Primer sequence
ttttttttttaatgatacggcgaccaccga

SEQ ID NO: 3 - DNA, 21 bp, Artificial Sequence
  Primer sequence
caagcagaagacggcatacga

SEQ ID NO: 4 - DNA, 20 bp, Artificial Sequence
  Primer sequence
aatgatacggcgaccaccga

SEQ ID NO: 5 - DNA, 20 bp, Artificial Sequence
  Primer target sequence
tcggtggtcgccgtatcatt

SEQ ID NO: 6 - DNA, 21 bp, Artificial Sequence
  Primer target sequence
tcgtatgccgtcttctgcttg

SEQ ID NO: 7 - DNA, 22 bp, Artificial Sequence
  Primer sequence
ttaatgatacggcgaccaccga

SEQ ID NO: 8 - DNA, 25 bp, Artificial Sequence
  Primer sequence
tttttaatgatacggcgaccaccga

SEQ ID NO: 9 - DNA, 40 bp, Artificial Sequence
  Primer sequence
ttttttttttttttttttttaatgatacggcgaccaccga